European Patent Application EP 4 140 475 A1, published March 1, 2023. Title: Synthetic virus-like lipoparticles. Applicant: Max-Planck-Gesellschaft zur Foerderung der Wissenschaften e.V. The sequence listing filed with the application follows.

SEQUENCE LISTING (35 sequences)

SEQ ID NO: 1 - protein, 1213 aa, SARS-CoV-2
  MISC_FEATURE (1)..(14): Signal peptide
  MISC_FEATURE (15)..(685): S1 Subunit
  MISC_FEATURE (319)..(541): Receptor Binding Site
  MISC_FEATURE (686)..(1213): S2 Subunit
MFVFLVLLPLVSSQCVNLTTRTQLPPAYTNSFTRGVYYPDKVFRSSVLHSTQDLFLPFFSNVTWFHAIHVSGTNGTKRFDNPVLPFNDGVYFASTEKSNIIRGWIFGTTLDSKTQSLLIVNNATNVVIKVCEFQFCNDPFLGVYYHKNNKSWMESEFRVYSSANNCTFEYVSQPFLMDLEGKQGNFKNLREFVFKNIDGYFKIYSKHTPINLVRDLPQGFSALEPLVDLPIGINITRFQTLLALHRSYLTPGDSSSGWTAGAAAYYVGYLQPRTFLLKYNENGTITDAVDCALDPLSETKCTLKSFTVEKGIYQTSNFRVQPTESIVRFPNITNLCPFGEVFNATRFASVYAWNRKRISNCVADYSVLYNSASFSTFKCYGVSPTKLNDLCFTNVYADSFVIRGDEVRQIAPGQTGKIADYNYKLPDDFTGCVIAWNSNNLDSKVGGNYNYLYRLFRKSNLKPFERDISTEIYQAGSTPCNGVEGFNCYFPLQSYGFQPTNGVGYQPYRVVVLSFELLHAPATVCGPKKSTNLVKNKCVNFNFNGLTGTGVLTESNKKFLPFQQFGRDIADTTDAVRDPQTLEILDITPCSFGGVSVITPGTNTSNQVAVLYQDVNCTEVPVAIHADQLTPTWRVYSTGSNVFQTRAGCLIGAEHVNNSYECDIPIGAGICASYQTQTNSPRRARSVASQSIIAYTMSLGAENSVAYSNNSIAIPTNFTISVTTEILPVSMTKTSVDCTMYICGDSTECSNLLLQYGSFCTQLNRALTGIAVEQDKNTQEVFAQVKQIYKTPPIKDFGGFNFSQILPDPSKPSKRSFIEDLLFNKVTLADAGFIKQYGDCLGDIAARDLICAQKFNGLTVLPPLLTDEMIAQYTSALLAGTITSGWTFGAGAALQIPFAMQMAYRFNGIGVTQNVLYENQKLIANQFNSAIGKIQDSLSSTASALGKLQDVVNQNAQALNTLVKQLSSNFGAISSVLNDILSRLDKVEAEVQIDRLITGRLQSLQTYVTQQLIRAAEIRASANLAATKMSECVLGQSKRVDFCGKGYHLMSFPQSAPHGVVFLHVTYVPAQEKNFTTAPAICHDGKAHFPREGVFVSNGTHWFVTQRNFYEPQIITTDNTFVSGNCDVVIGIVNNTVYDPLQPELDSFKEELDKYFKNHTSPDVDLGDISGINASVVNIQKEIDRLNEVAKNLNESLIDLQELGKYEQYIKWP

SEQ ID NO: 2 - protein, 1242 aa, Unknown
  native SARS-CoV-2 Spike ectodomain protein construct
  MISC_FEATURE (668)..(668): furin cleavage site RRAR replaced by A
  Site (1197)..(1202): C-terminal thrombin cleavage site
  MISC_FEATURE (1203)..(1236): T4 foldon trimerization domain
  MISC_FEATURE (1237)..(1242): hexa-His tag
CVNLTTRTQLPPAYTNSFTRGVYYPDKVFRSSVLHSTQDLFLPFFSNVTWFHAIHVSGTNGTKRFDNPVLPFNDGVYFASTEKSNIIRGWIFGTTLDSKTQSLLIVNNATNVVIKVCEFQFCNDPFLGVYYHKNNKSWMESEFRVYSSANNCTFEYVSQPFLMDLEGKQGNFKNLREFVFKNIDGYFKIYSKHTPINLVRDLPQGFSALEPLVDLPIGINITRFQTLLALHRSYLTPGDSSSGWTAGAAAYYVGYLQPRTFLLKYNENGTITDAVDCALDPLSETKCTLKSFTVEKGIYQTSNFRVQPTESIVRFPNITNLCPFGEVFNATRFASVYAWNRKRISNCVADYSVLYNSASFSTFKCYGVSPTKLNDLCFTNVYADSFVIRGDEVRQIAPGQTGKIADYNYKLPDDFTGCVIAWNSNNLDSKVGGNYNYLYRLFRKSNLKPFERDISTEIYQAGSTPCNGVEGFNCYFPLQSYGFQPTNGVGYQPYRVVVLSFELLHAPATVCGPKKSTNLVKNKCVNFNFNGLTGTGVLTESNKKFLPFQQFGRDIADTTDAVRDPQTLEILDITPCSFGGVSVITPGTNTSNQVAVLYQDVNCTEVPVAIHADQLTPTWRVYSTGSNVFQTRAGCLIGAEHVNNSYECDIPIGAGICASYQTQTNSPASVASQSIIAYTMSLGAENSVAYSNNSIAIPTNFTISVTTEILPVSMTKTSVDCTMYICGDSTECSNLLLQYGSFCTQLNRALTGIAVEQDKNTQEVFAQVKQIYKTPPIKDFGGFNFSQILPDPSKPSKRSFIEDLLFNKVTLADAGFIKQYGDCLGDIAARDLICAQKFNGLTVLPPLLTDEMIAQYTSALLAGTITSGWTFGAGAALQIPFAMQMAYRFNGIGVTQNVLYENQKLIANQFNSAIGKIQDSLSSTASALGKLQDVVNQNAQALNTLVKQLSSNFGAISSVLNDILSRLDKVEAEVQIDRLITGRLQSLQTYVTQQLIRAAEIRASANLAATKMSECVLGQSKRVDFCGKGYHLMSFPQSAPHGVVFLHVTYVPAQEKNFTTAPAICHDGKAHFPREGVFVSNGTHWFVTQRNFYEPQIITTDNTFVSGNCDVVIGIVNNTVYDPLQPELDSFKEELDKYFKNHTSPDVDLGDISGINASVVNIQKEIDRLNEVAKNLNESLIDLQELGKYEQYIKWPSGRLVPRGSPGSGYIPEAPRDGQAYVRKDGEWVLLSTFLGHHHHHH

SEQ ID NO: 3 - protein, 6 aa, Unknown
  C-terminal thrombin cleavage site
SGRLVP

SEQ ID NO: 4 - protein, 34 aa, Unknown
  T4 foldon trimerization domain
RGSPGSGYIPEAPRDGQAYVRKDGEWVLLSTFLG

SEQ ID NO: 5 - protein, 1196 aa, Unknown
  SARS-CoV-2 Spike protein native ectodomain
CVNLTTRTQLPPAYTNSFTRGVYYPDKVFRSSVLHSTQDLFLPFFSNVTWFHAIHVSGTNGTKRFDNPVLPFNDGVYFASTEKSNIIRGWIFGTTLDSKTQSLLIVNNATNVVIKVCEFQFCNDPFLGVYYHKNNKSWMESEFRVYSSANNCTFEYVSQPFLMDLEGKQGNFKNLREFVFKNIDGYFKIYSKHTPINLVRDLPQGFSALEPLVDLPIGINITRFQTLLALHRSYLTPGDSSSGWTAGAAAYYVGYLQPRTFLLKYNENGTITDAVDCALDPLSETKCTLKSFTVEKGIYQTSNFRVQPTESIVRFPNITNLCPFGEVFNATRFASVYAWNRKRISNCVADYSVLYNSASFSTFKCYGVSPTKLNDLCFTNVYADSFVIRGDEVRQIAPGQTGKIADYNYKLPDDFTGCVIAWNSNNLDSKVGGNYNYLYRLFRKSNLKPFERDISTEIYQAGSTPCNGVEGFNCYFPLQSYGFQPTNGVGYQPYRVVVLSFELLHAPATVCGPKKSTNLVKNKCVNFNFNGLTGTGVLTESNKKFLPFQQFGRDIADTTDAVRDPQTLEILDITPCSFGGVSVITPGTNTSNQVAVLYQDVNCTEVPVAIHADQLTPTWRVYSTGSNVFQTRAGCLIGAEHVNNSYECDIPIGAGICASYQTQTNSPASVASQSIIAYTMSLGAENSVAYSNNSIAIPTNFTISVTTEILPVSMTKTSVDCTMYICGDSTECSNLLLQYGSFCTQLNRALTGIAVEQDKNTQEVFAQVKQIYKTPPIKDFGGFNFSQILPDPSKPSKRSFIEDLLFNKVTLADAGFIKQYGDCLGDIAARDLICAQKFNGLTVLPPLLTDEMIAQYTSALLAGTITSGWTFGAGAALQIPFAMQMAYRFNGIGVTQNVLYENQKLIANQFNSAIGKIQDSLSSTASALGKLQDVVNQNAQALNTLVKQLSSNFGAISSVLNDILSRLDKVEAEVQIDRLITGRLQSLQTYVTQQLIRAAEIRASANLAATKMSECVLGQSKRVDFCGKGYHLMSFPQSAPHGVVFLHVTYVPAQEKNFTTAPAICHDGKAHFPREGVFVSNGTHWFVTQRNFYEPQIITTDNTFVSGNCDVVIGIVNNTVYDPLQPELDSFKEELDKYFKNHTSPDVDLGDISGINASVVNIQKEIDRLNEVAKNLNESLIDLQELGKYEQYIKWP

SEQ ID NO: 6 - protein, 1196 aa, Unknown
  SARS-CoV-2 Spike protein native ectodomain L4F mutant
CVNFTTRTQLPPAYTNSFTRGVYYPDKVFRSSVLHSTQDLFLPFFSNVTWFHAIHVSGTNGTKRFDNPVLPFNDGVYFASTEKSNIIRGWIFGTTLDSKTQSLLIVNNATNVVIKVCEFQFCNDPFLGVYYHKNNKSWMESEFRVYSSANNCTFEYVSQPFLMDLEGKQGNFKNLREFVFKNIDGYFKIYSKHTPINLVRDLPQGFSALEPLVDLPIGINITRFQTLLALHRSYLTPGDSSSGWTAGAAAYYVGYLQPRTFLLKYNENGTITDAVDCALDPLSETKCTLKSFTVEKGIYQTSNFRVQPTESIVRFPNITNLCPFGEVFNATRFASVYAWNRKRISNCVADYSVLYNSASFSTFKCYGVSPTKLNDLCFTNVYADSFVIRGDEVRQIAPGQTGKIADYNYKLPDDFTGCVIAWNSNNLDSKVGGNYNYLYRLFRKSNLKPFERDISTEIYQAGSTPCNGVEGFNCYFPLQSYGFQPTNGVGYQPYRVVVLSFELLHAPATVCGPKKSTNLVKNKCVNFNFNGLTGTGVLTESNKKFLPFQQFGRDIADTTDAVRDPQTLEILDITPCSFGGVSVITPGTNTSNQVAVLYQDVNCTEVPVAIHADQLTPTWRVYSTGSNVFQTRAGCLIGAEHVNNSYECDIPIGAGICASYQTQTNSPASVASQSIIAYTMSLGAENSVAYSNNSIAIPTNFTISVTTEILPVSMTKTSVDCTMYICGDSTECSNLLLQYGSFCTQLNRALTGIAVEQDKNTQEVFAQVKQIYKTPPIKDFGGFNFSQILPDPSKPSKRSFIEDLLFNKVTLADAGFIKQYGDCLGDIAARDLICAQKFNGLTVLPPLLTDEMIAQYTSALLAGTITSGWTFGAGAALQIPFAMQMAYRFNGIGVTQNVLYENQKLIANQFNSAIGKIQDSLSSTASALGKLQDVVNQNAQALNTLVKQLSSNFGAISSVLNDILSRLDKVEAEVQIDRLITGRLQSLQTYVTQQLIRAAEIRASANLAATKMSECVLGQSKRVDFCGKGYHLMSFPQSAPHGVVFLHVTYVPAQEKNFTTAPAICHDGKAHFPREGVFVSNGTHWFVTQRNFYEPQIITTDNTFVSGNCDVVIGIVNNTVYDPLQPELDSFKEELDKYFKNHTSPDVDLGDISGINASVVNIQKEIDRLNEVAKNLNESLIDLQELGKYEQYIKWP

SEQ ID NO: 7 - protein, 1196 aa, Unknown
  SARS-CoV-2 Spike protein native ectodomain T6N mutant
CVNLTNRTQLPPAYTNSFTRGVYYPDKVFRSSVLHSTQDLFLPFFSNVTWFHAIHVSGTNGTKRFDNPVLPFNDGVYFASTEKSNIIRGWIFGTTLDSKTQSLLIVNNATNVVIKVCEFQFCNDPFLGVYYHKNNKSWMESEFRVYSSANNCTFEYVSQPFLMDLEGKQGNFKNLREFVFKNIDGYFKIYSKHTPINLVRDLPQGFSALEPLVDLPIGINITRFQTLLALHRSYLTPGDSSSGWTAGAAAYYVGYLQPRTFLLKYNENGTITDAVDCALDPLSETKCTLKSFTVEKGIYQTSNFRVQPTESIVRFPNITNLCPFGEVFNATRFASVYAWNRKRISNCVADYSVLYNSASFSTFKCYGVSPTKLNDLCFTNVYADSFVIRGDEVRQIAPGQTGKIADYNYKLPDDFTGCVIAWNSNNLDSKVGGNYNYLYRLFRKSNLKPFERDISTEIYQAGSTPCNGVEGFNCYFPLQSYGFQPTNGVGYQPYRVVVLSFELLHAPATVCGPKKSTNLVKNKCVNFNFNGLTGTGVLTESNKKFLPFQQFGRDIADTTDAVRDPQTLEILDITPCSFGGVSVITPGTNTSNQVAVLYQDVNCTEVPVAIHADQLTPTWRVYSTGSNVFQTRAGCLIGAEHVNNSYECDIPIGAGICASYQTQTNSPASVASQSIIAYTMSLGAENSVAYSNNSIAIPTNFTISVTTEILPVSMTKTSVDCTMYICGDSTECSNLLLQYGSFCTQLNRALTGIAVEQDKNTQEVFAQVKQIYKTPPIKDFGGFNFSQILPDPSKPSKRSFIEDLLFNKVTLADAGFIKQYGDCLGDIAARDLICAQKFNGLTVLPPLLTDEMIAQYTSALLAGTITSGWTFGAGAALQIPFAMQMAYRFNGIGVTQNVLYENQKLIANQFNSAIGKIQDSLSSTASALGKLQDVVNQNAQALNTLVKQLSSNFGAISSVLNDILSRLDKVEAEVQIDRLITGRLQSLQTYVTQQLIRAAEIRASANLAATKMSECVLGQSKRVDFCGKGYHLMSFPQSAPHGVVFLHVTYVPAQEKNFTTAPAICHDGKAHFPREGVFVSNGTHWFVTQRNFYEPQIITTDNTFVSGNCDVVIGIVNNTVYDPLQPELDSFKEELDKYFKNHTSPDVDLGDISGINASVVNIQKEIDRLNEVAKNLNESLIDLQELGKYEQYIKWP

SEQ ID NO: 8 - protein, 1196 aa, Unknown
  SARS-CoV-2 Spike protein native ectodomain P12S mutant
CVNLTTRTQLPSAYTNSFTRGVYYPDKVFRSSVLHSTQDLFLPFFSNVTWFHAIHVSGTNGTKRFDNPVLPFNDGVYFASTEKSNIIRGWIFGTTLDSKTQSLLIVNNATNVVIKVCEFQFCNDPFLGVYYHKNNKSWMESEFRVYSSANNCTFEYVSQPFLMDLEGKQGNFKNLREFVFKNIDGYFKIYSKHTPINLVRDLPQGFSALEPLVDLPIGINITRFQTLLALHRSYLTPGDSSSGWTAGAAAYYVGYLQPRTFLLKYNENGTITDAVDCALDPLSETKCTLKSFTVEKGIYQTSNFRVQPTESIVRFPNITNLCPFGEVFNATRFASVYAWNRKRISNCVADYSVLYNSASFSTFKCYGVSPTKLNDLCFTNVYADSFVIRGDEVRQIAPGQTGKIADYNYKLPDDFTGCVIAWNSNNLDSKVGGNYNYLYRLFRKSNLKPFERDISTEIYQAGSTPCNGVEGFNCYFPLQSYGFQPTNGVGYQPYRVVVLSFELLHAPATVCGPKKSTNLVKNKCVNFNFNGLTGTGVLTESNKKFLPFQQFGRDIADTTDAVRDPQTLEILDITPCSFGGVSVITPGTNTSNQVAVLYQDVNCTEVPVAIHADQLTPTWRVYSTGSNVFQTRAGCLIGAEHVNNSYECDIPIGAGICASYQTQTNSPASVASQSIIAYTMSLGAENSVAYSNNSIAIPTNFTISVTTEILPVSMTKTSVDCTMYICGDSTECSNLLLQYGSFCTQLNRALTGIAVEQDKNTQEVFAQVKQIYKTPPIKDFGGFNFSQILPDPSKPSKRSFIEDLLFNKVTLADAGFIKQYGDCLGDIAARDLICAQKFNGLTVLPPLLTDEMIAQYTSALLAGTITSGWTFGAGAALQIPFAMQMAYRFNGIGVTQNVLYENQKLIANQFNSAIGKIQDSLSSTASALGKLQDVVNQNAQALNTLVKQLSSNFGAISSVLNDILSRLDKVEAEVQIDRLITGRLQSLQTYVTQQLIRAAEIRASANLAATKMSECVLGQSKRVDFCGKGYHLMSFPQSAPHGVVFLHVTYVPAQEKNFTTAPAICHDGKAHFPREGVFVSNGTHWFVTQRNFYEPQIITTDNTFVSGNCDVVIGIVNNTVYDPLQPELDSFKEELDKYFKNHTSPDVDLGDISGINASVVNIQKEIDRLNEVAKNLNESLIDLQELGKYEQYIKWP

SEQ ID NO: 9 - protein, 1196 aa, Unknown
  SARS-CoV-2 Spike protein native ectodomain D66A mutant
CVNLTTRTQLPPAYTNSFTRGVYYPDKVFRSSVLHSTQDLFLPFFSNVTWFHAIHVSGTNGTKRFANPVLPFNDGVYFASTEKSNIIRGWIFGTTLDSKTQSLLIVNNATNVVIKVCEFQFCNDPFLGVYYHKNNKSWMESEFRVYSSANNCTFEYVSQPFLMDLEGKQGNFKNLREFVFKNIDGYFKIYSKHTPINLVRDLPQGFSALEPLVDLPIGINITRFQTLLALHRSYLTPGDSSSGWTAGAAAYYVGYLQPRTFLLKYNENGTITDAVDCALDPLSETKCTLKSFTVEKGIYQTSNFRVQPTESIVRFPNITNLCPFGEVFNATRFASVYAWNRKRISNCVADYSVLYNSASFSTFKCYGVSPTKLNDLCFTNVYADSFVIRGDEVRQIAPGQTGKIADYNYKLPDDFTGCVIAWNSNNLDSKVGGNYNYLYRLFRKSNLKPFERDISTEIYQAGSTPCNGVEGFNCYFPLQSYGFQPTNGVGYQPYRVVVLSFELLHAPATVCGPKKSTNLVKNKCVNFNFNGLTGTGVLTESNKKFLPFQQFGRDIADTTDAVRDPQTLEILDITPCSFGGVSVITPGTNTSNQVAVLYQDVNCTEVPVAIHADQLTPTWRVYSTGSNVFQTRAGCLIGAEHVNNSYECDIPIGAGICASYQTQTNSPASVASQSIIAYTMSLGAENSVAYSNNSIAIPTNFTISVTTEILPVSMTKTSVDCTMYICGDSTECSNLLLQYGSFCTQLNRALTGIAVEQDKNTQEVFAQVKQIYKTPPIKDFGGFNFSQILPDPSKPSKRSFIEDLLFNKVTLADAGFIKQYGDCLGDIAARDLICAQKFNGLTVLPPLLTDEMIAQYTSALLAGTITSGWTFGAGAALQIPFAMQMAYRFNGIGVTQNVLYENQKLIANQFNSAIGKIQDSLSSTASALGKLQDVVNQNAQALNTLVKQLSSNFGAISSVLNDILSRLDKVEAEVQIDRLITGRLQSLQTYVTQQLIRAAEIRASANLAATKMSECVLGQSKRVDFCGKGYHLMSFPQSAPHGVVFLHVTYVPAQEKNFTTAPAICHDGKAHFPREGVFVSNGTHWFVTQRNFYEPQIITTDNTFVSGNCDVVIGIVNNTVYDPLQPELDSFKEELDKYFKNHTSPDVDLGDISGINASVVNIQKEIDRLNEVAKNLNESLIDLQELGKYEQYIKWP

SEQ ID NO: 10 - protein, 1196 aa, Unknown
  SARS-CoV-2 Spike protein native ectodomain D124Y mutant
CVNLTTRTQLPPAYTNSFTRGVYYPDKVFRSSVLHSTQDLFLPFFSNVTWFHAIHVSGTNGTKRFDNPVLPFNDGVYFASTEKSNIIRGWIFGTTLDSKTQSLLIVNNATNVVIKVCEFQFCNYPFLGVYYHKNNKSWMESEFRVYSSANNCTFEYVSQPFLMDLEGKQGNFKNLREFVFKNIDGYFKIYSKHTPINLVRDLPQGFSALEPLVDLPIGINITRFQTLLALHRSYLTPGDSSSGWTAGAAAYYVGYLQPRTFLLKYNENGTITDAVDCALDPLSETKCTLKSFTVEKGIYQTSNFRVQPTESIVRFPNITNLCPFGEVFNATRFASVYAWNRKRISNCVADYSVLYNSASFSTFKCYGVSPTKLNDLCFTNVYADSFVIRGDEVRQIAPGQTGKIADYNYKLPDDFTGCVIAWNSNNLDSKVGGNYNYLYRLFRKSNLKPFERDISTEIYQAGSTPCNGVEGFNCYFPLQSYGFQPTNGVGYQPYRVVVLSFELLHAPATVCGPKKSTNLVKNKCVNFNFNGLTGTGVLTESNKKFLPFQQFGRDIADTTDAVRDPQTLEILDITPCSFGGVSVITPGTNTSNQVAVLYQDVNCTEVPVAIHADQLTPTWRVYSTGSNVFQTRAGCLIGAEHVNNSYECDIPIGAGICASYQTQTNSPASVASQSIIAYTMSLGAENSVAYSNNSIAIPTNFTISVTTEILPVSMTKTSVDCTMYICGDSTECSNLLLQYGSFCTQLNRALTGIAVEQDKNTQEVFAQVKQIYKTPPIKDFGGFNFSQILPDPSKPSKRSFIEDLLFNKVTLADAGFIKQYGDCLGDIAARDLICAQKFNGLTVLPPLLTDEMIAQYTSALLAGTITSGWTFGAGAALQIPFAMQMAYRFNGIGVTQNVLYENQKLIANQFNSAIGKIQDSLSSTASALGKLQDVVNQNAQALNTLVKQLSSNFGAISSVLNDILSRLDKVEAEVQIDRLITGRLQSLQTYVTQQLIRAAEIRASANLAATKMSECVLGQSKRVDFCGKGYHLMSFPQSAPHGVVFLHVTYVPAQEKNFTTAPAICHDGKAHFPREGVFVSNGTHWFVTQRNFYEPQIITTDNTFVSGNCDVVIGIVNNTVYDPLQPELDSFKEELDKYFKNHTSPDVDLGDISGINASVVNIQKEIDRLNEVAKNLNESLIDLQELGKYEQYIKWP

SEQ ID NO: 11 - protein, 1196 aa, Unknown
  SARS-CoV-2 Spike protein native ectodomain R176S mutant
CVNLTTRTQLPPAYTNSFTRGVYYPDKVFRSSVLHSTQDLFLPFFSNVTWFHAIHVSGTNGTKRFDNPVLPFNDGVYFASTEKSNIIRGWIFGTTLDSKTQSLLIVNNATNVVIKVCEFQFCNDPFLGVYYHKNNKSWMESEFRVYSSANNCTFEYVSQPFLMDLEGKQGNFKNLSEFVFKNIDGYFKIYSKHTPINLVRDLPQGFSALEPLVDLPIGINITRFQTLLALHRSYLTPGDSSSGWTAGAAAYYVGYLQPRTFLLKYNENGTITDAVDCALDPLSETKCTLKSFTVEKGIYQTSNFRVQPTESIVRFPNITNLCPFGEVFNATRFASVYAWNRKRISNCVADYSVLYNSASFSTFKCYGVSPTKLNDLCFTNVYADSFVIRGDEVRQIAPGQTGKIADYNYKLPDDFTGCVIAWNSNNLDSKVGGNYNYLYRLFRKSNLKPFERDISTEIYQAGSTPCNGVEGFNCYFPLQSYGFQPTNGVGYQPYRVVVLSFELLHAPATVCGPKKSTNLVKNKCVNFNFNGLTGTGVLTESNKKFLPFQQFGRDIADTTDAVRDPQTLEILDITPCSFGGVSVITPGTNTSNQVAVLYQDVNCTEVPVAIHADQLTPTWRVYSTGSNVFQTRAGCLIGAEHVNNSYECDIPIGAGICASYQTQTNSPASVASQSIIAYTMSLGAENSVAYSNNSIAIPTNFTISVTTEILPVSMTKTSVDCTMYICGDSTECSNLLLQYGSFCTQLNRALTGIAVEQDKNTQEVFAQVKQIYKTPPIKDFGGFNFSQILPDPSKPSKRSFIEDLLFNKVTLADAGFIKQYGDCLGDIAARDLICAQKFNGLTVLPPLLTDEMIAQYTSALLAGTITSGWTFGAGAALQIPFAMQMAYRFNGIGVTQNVLYENQKLIANQFNSAIGKIQDSLSSTASALGKLQDVVNQNAQALNTLVKQLSSNFGAISSVLNDILSRLDKVEAEVQIDRLITGRLQSLQTYVTQQLIRAAEIRASANLAATKMSECVLGQSKRVDFCGKGYHLMSFPQSAPHGVVFLHVTYVPAQEKNFTTAPAICHDGKAHFPREGVFVSNGTHWFVTQRNFYEPQIITTDNTFVSGNCDVVIGIVNNTVYDPLQPELDSFKEELDKYFKNHTSPDVDLGDISGINASVVNIQKEIDRLNEVAKNLNESLIDLQELGKYEQYIKWP

SEQ ID NO: 12 - protein, 1196 aa, Unknown
  SARS-CoV-2 Spike protein native ectodomain D201G mutant
CVNLTTRTQLPPAYTNSFTRGVYYPDKVFRSSVLHSTQDLFLPFFSNVTWFHAIHVSGTNGTKRFDNPVLPFNDGVYFASTEKSNIIRGWIFGTTLDSKTQSLLIVNNATNVVIKVCEFQFCNDPFLGVYYHKNNKSWMESEFRVYSSANNCTFEYVSQPFLMDLEGKQGNFKNLREFVFKNIDGYFKIYSKHTPINLVRGLPQGFSALEPLVDLPIGINITRFQTLLALHRSYLTPGDSSSGWTAGAAAYYVGYLQPRTFLLKYNENGTITDAVDCALDPLSETKCTLKSFTVEKGIYQTSNFRVQPTESIVRFPNITNLCPFGEVFNATRFASVYAWNRKRISNCVADYSVLYNSASFSTFKCYGVSPTKLNDLCFTNVYADSFVIRGDEVRQIAPGQTGKIADYNYKLPDDFTGCVIAWNSNNLDSKVGGNYNYLYRLFRKSNLKPFERDISTEIYQAGSTPCNGVEGFNCYFPLQSYGFQPTNGVGYQPYRVVVLSFELLHAPATVCGPKKSTNLVKNKCVNFNFNGLTGTGVLTESNKKFLPFQQFGRDIADTTDAVRDPQTLEILDITPCSFGGVSVITPGTNTSNQVAVLYQDVNCTEVPVAIHADQLTPTWRVYSTGSNVFQTRAGCLIGAEHVNNSYECDIPIGAGICASYQTQTNSPASVASQSIIAYTMSLGAENSVAYSNNSIAIPTNFTISVTTEILPVSMTKTSVDCTMYICGDSTECSNLLLQYGSFCTQLNRALTGIAVEQDKNTQEVFAQVKQIYKTPPIKDFGGFNFSQILPDPSKPSKRSFIEDLLFNKVTLADAGFIKQYGDCLGDIAARDLICAQKFNGLTVLPPLLTDEMIAQYTSALLAGTITSGWTFGAGAALQIPFAMQMAYRFNGIGVTQNVLYENQKLIANQFNSAIGKIQDSLSSTASALGKLQDVVNQNAQALNTLVKQLSSNFGAISSVLNDILSRLDKVEAEVQIDRLITGRLQSLQTYVTQQLIRAAEIRASANLAATKMSECVLGQSKRVDFCGKGYHLMSFPQSAPHGVVFLHVTYVPAQEKNFTTAPAICHDGKAHFPREGVFVSNGTHWFVTQRNFYEPQIITTDNTFVSGNCDVVIGIVNNTVYDPLQPELDSFKEELDKYFKNHTSPDVDLGDISGINASVVNIQKEIDRLNEVAKNLNESLIDLQELGKYEQYIKWP

SEQ ID NO: 13 - protein, 1196 aa, Unknown
  SARS-CoV-2 Spike protein native ectodomain R232I mutant
CVNLTTRTQLPPAYTNSFTRGVYYPDKVFRSSVLHSTQDLFLPFFSNVTWFHAIHVSGTNGTKRFDNPVLPFNDGVYFASTEKSNIIRGWIFGTTLDSKTQSLLIVNNATNVVIKVCEFQFCNDPFLGVYYHKNNKSWMESEFRVYSSANNCTFEYVSQPFLMDLEGKQGNFKNLREFVFKNIDGYFKIYSKHTPINLVRDLPQGFSALEPLVDLPIGINITRFQTLLALHISYLTPGDSSSGWTAGAAAYYVGYLQPRTFLLKYNENGTITDAVDCALDPLSETKCTLKSFTVEKGIYQTSNFRVQPTESIVRFPNITNLCPFGEVFNATRFASVYAWNRKRISNCVADYSVLYNSASFSTFKCYGVSPTKLNDLCFTNVYADSFVIRGDEVRQIAPGQTGKIADYNYKLPDDFTGCVIAWNSNNLDSKVGGNYNYLYRLFRKSNLKPFERDISTEIYQAGSTPCNGVEGFNCYFPLQSYGFQPTNGVGYQPYRVVVLSFELLHAPATVCGPKKSTNLVKNKCVNFNFNGLTGTGVLTESNKKFLPFQQFGRDIADTTDAVRDPQTLEILDITPCSFGGVSVITPGTNTSNQVAVLYQDVNCTEVPVAIHADQLTPTWRVYSTGSNVFQTRAGCLIGAEHVNNSYECDIPIGAGICASYQTQTNSPASVASQSIIAYTMSLGAENSVAYSNNSIAIPTNFTISVTTEILPVSMTKTSVDCTMYICGDSTECSNLLLQYGSFCTQLNRALTGIAVEQDKNTQEVFAQVKQIYKTPPIKDFGGFNFSQILPDPSKPSKRSFIEDLLFNKVTLADAGFIKQYGDCLGDIAARDLICAQKFNGLTVLPPLLTDEMIAQYTSALLAGTITSGWTFGAGAALQIPFAMQMAYRFNGIGVTQNVLYENQKLIANQFNSAIGKIQDSLSSTASALGKLQDVVNQNAQALNTLVKQLSSNFGAISSVLNDILSRLDKVEAEVQIDRLITGRLQSLQTYVTQQLIRAAEIRASANLAATKMSECVLGQSKRVDFCGKGYHLMSFPQSAPHGVVFLHVTYVPAQEKNFTTAPAICHDGKAHFPREGVFVSNGTHWFVTQRNFYEPQIITTDNTFVSGNCDVVIGIVNNTVYDPLQPELDSFKEELDKYFKNHTSPDVDLGDISGINASVVNIQKEIDRLNEVAKNLNESLIDLQELGKYEQYIKWP

SEQ ID NO: 14 - protein, 1196 aa, Unknown
  SARS-CoV-2 Spike protein native ectodomain K403N mutant
CVNLTTRTQLPPAYTNSFTRGVYYPDKVFRSSVLHSTQDLFLPFFSNVTWFHAIHVSGTNGTKRFDNPVLPFNDGVYFASTEKSNIIRGWIFGTTLDSKTQSLLIVNNATNVVIKVCEFQFCNDPFLGVYYHKNNKSWMESEFRVYSSANNCTFEYVSQPFLMDLEGKQGNFKNLREFVFKNIDGYFKIYSKHTPINLVRDLPQGFSALEPLVDLPIGINITRFQTLLALHRSYLTPGDSSSGWTAGAAAYYVGYLQPRTFLLKYNENGTITDAVDCALDPLSETKCTLKSFTVEKGIYQTSNFRVQPTESIVRFPNITNLCPFGEVFNATRFASVYAWNRKRISNCVADYSVLYNSASFSTFKCYGVSPTKLNDLCFTNVYADSFVIRGDEVRQIAPGQTGNIADYNYKLPDDFTGCVIAWNSNNLDSKVGGNYNYLYRLFRKSNLKPFERDISTEIYQAGSTPCNGVEGFNCYFPLQSYGFQPTNGVGYQPYRVVVLSFELLHAPATVCGPKKSTNLVKNKCVNFNFNGLTGTGVLTESNKKFLPFQQFGRDIADTTDAVRDPQTLEILDITPCSFGGVSVITPGTNTSNQVAVLYQDVNCTEVPVAIHADQLTPTWRVYSTGSNVFQTRAGCLIGAEHVNNSYECDIPIGAGICASYQTQTNSPASVASQSIIAYTMSLGAENSVAYSNNSIAIPTNFTISVTTEILPVSMTKTSVDCTMYICGDSTECSNLLLQYGSFCTQLNRALTGIAVEQDKNTQEVFAQVKQIYKTPPIKDFGGFNFSQILPDPSKPSKRSFIEDLLFNKVTLADAGFIKQYGDCLGDIAARDLICAQKFNGLTVLPPLLTDEMIAQYTSALLAGTITSGWTFGAGAALQIPFAMQMAYRFNGIGVTQNVLYENQKLIANQFNSAIGKIQDSLSSTASALGKLQDVVNQNAQALNTLVKQLSSNFGAISSVLNDILSRLDKVEAEVQIDRLITGRLQSLQTYVTQQLIRAAEIRASANLAATKMSECVLGQSKRVDFCGKGYHLMSFPQSAPHGVVFLHVTYVPAQEKNFTTAPAICHDGKAHFPREGVFVSNGTHWFVTQRNFYEPQIITTDNTFVSGNCDVVIGIVNNTVYDPLQPELDSFKEELDKYFKNHTSPDVDLGDISGINASVVNIQKEIDRLNEVAKNLNESLIDLQELGKYEQYIKWP

SEQ ID NO: 15 - protein, 1196 aa, Unknown
  SARS-CoV-2 Spike protein native ectodomain K403T mutant
CVNLTTRTQLPPAYTNSFTRGVYYPDKVFRSSVLHSTQDLFLPFFSNVTWFHAIHVSGTNGTKRFDNPVLPFNDGVYFASTEKSNIIRGWIFGTTLDSKTQSLLIVNNATNVVIKVCEFQFCNDPFLGVYYHKNNKSWMESEFRVYSSANNCTFEYVSQPFLMDLEGKQGNFKNLREFVFKNIDGYFKIYSKHTPINLVRDLPQGFSALEPLVDLPIGINITRFQTLLALHRSYLTPGDSSSGWTAGAAAYYVGYLQPRTFLLKYNENGTITDAVDCALDPLSETKCTLKSFTVEKGIYQTSNFRVQPTESIVRFPNITNLCPFGEVFNATRFASVYAWNRKRISNCVADYSVLYNSASFSTFKCYGVSPTKLNDLCFTNVYADSFVIRGDEVRQIAPGQTGTIADYNYKLPDDFTGCVIAWNSNNLDSKVGGNYNYLYRLFRKSNLKPFERDISTEIYQAGSTPCNGVEGFNCYFPLQSYGFQPTNGVGYQPYRVVVLSFELLHAPATVCGPKKSTNLVKNKCVNFNFNGLTGTGVLTESNKKFLPFQQFGRDIADTTDAVRDPQTLEILDITPCSFGGVSVITPGTNTSNQVAVLYQDVNCTEVPVAIHADQLTPTWRVYSTGSNVFQTRAGCLIGAEHVNNSYECDIPIGAGICASYQTQTNSPASVASQSIIAYTMSLGAENSVAYSNNSIAIPTNFTISVTTEILPVSMTKTSVDCTMYICGDSTECSNLLLQYGSFCTQLNRALTGIAVEQDKNTQEVFAQVKQIYKTPPIKDFGGFNFSQILPDPSKPSKRSFIEDLLFNKVTLADAGFIKQYGDCLGDIAARDLICAQKFNGLTVLPPLLTDEMIAQYTSALLAGTITSGWTFGAGAALQIPFAMQMAYRFNGIGVTQNVLYENQKLIANQFNSAIGKIQDSLSSTASALGKLQDVVNQNAQALNTLVKQLSSNFGAISSVLNDILSRLDKVEAEVQIDRLITGRLQSLQTYVTQQLIRAAEIRASANLAATKMSECVLGQSKRVDFCGKGYHLMSFPQSAPHGVVFLHVTYVPAQEKNFTTAPAICHDGKAHFPREGVFVSNGTHWFVTQRNFYEPQIITTDNTFVSGNCDVVIGIVNNTVYDPLQPELDSFKEELDKYFKNHTSPDVDLGDISGINASVVNIQKEIDRLNEVAKNLNESLIDLQELGKYEQYIKWP

SEQ ID NO: 16 - protein, 1196 aa, Unknown
  SARS-CoV-2 Spike protein native ectodomain L411R mutant
CVNLTTRTQLPPAYTNSFTRGVYYPDKVFRSSVLHSTQDLFLPFFSNVTWFHAIHVSGTNGTKRFDNPVLPFNDGVYFASTEKSNIIRGWIFGTTLDSKTQSLLIVNNATNVVIKVCEFQFCNDPFLGVYYHKNNKSWMESEFRVYSSANNCTFEYVSQPFLMDLEGKQGNFKNLREFVFKNIDGYFKIYSKHTPINLVRDLPQGFSALEPLVDLPIGINITRFQTLLALHRSYLTPGDSSSGWTAGAAAYYVGYLQPRTFLLKYNENGTITDAVDCALDPLSETKCTLKSFTVEKGIYQTSNFRVQPTESIVRFPNITNLCPFGEVFNATRFASVYAWNRKRISNCVADYSVLYNSASFSTFKCYGVSPTKLNDLCFTNVYADSFVIRGDEVRQIAPGQTGKIADYNYKRPDDFTGCVIAWNSNNLDSKVGGNYNYLYRLFRKSNLKPFERDISTEIYQAGSTPCNGVEGFNCYFPLQSYGFQPTNGVGYQPYRVVVLSFELLHAPATVCGPKKSTNLVKNKCVNFNFNGLTGTGVLTESNKKFLPFQQFGRDIADTTDAVRDPQTLEILDITPCSFGGVSVITPGTNTSNQVAVLYQDVNCTEVPVAIHADQLTPTWRVYSTGSNVFQTRAGCLIGAEHVNNSYECDIPIGAGICASYQTQTNSPASVASQSIIAYTMSLGAENSVAYSNNSIAIPTNFTISVTTEILPVSMTKTSVDCTMYICGDSTECSNLLLQYGSFCTQLNRALTGIAVEQDKNTQEVFAQVKQIYKTPPIKDFGGFNFSQILPDPSKPSKRSFIEDLLFNKVTLADAGFIKQYGDCLGDIAARDLICAQKFNGLTVLPPLLTDEMIAQYTSALLAGTITSGWTFGAGAALQIPFAMQMAYRFNGIGVTQNVLYENQKLIANQFNSAIGKIQDSLSSTASALGKLQDVVNQNAQALNTLVKQLSSNFGAISSVLNDILSRLDKVEAEVQIDRLITGRLQSLQTYVTQQLIRAAEIRASANLAATKMSECVLGQSKRVDFCGKGYHLMSFPQSAPHGVVFLHVTYVPAQEKNFTTAPAICHDGKAHFPREGVFVSNGTHWFVTQRNFYEPQIITTDNTFVSGNCDVVIGIVNNTVYDPLQPELDSFKEELDKYFKNHTSPDVDLGDISGINASVVNIQKEIDRLNEVAKNLNESLIDLQELGKYEQYIKWP

SEQ ID NO: 17 - protein, 1196 aa, Unknown
  SARS-CoV-2 Spike protein native ectodomain E470K mutant
CVNLTTRTQLPPAYTNSFTRGVYYPDKVFRSSVLHSTQDLFLPFFSNVTWFHAIHVSGTNGTKRFDNPVLPFNDGVYFASTEKSNIIRGWIFGTTLDSKTQSLLIVNNATNVVIKVCEFQFCNDPFLGVYYHKNNKSWMESEFRVYSSANNCTFEYVSQPFLMDLEGKQGNFKNLREFVFKNIDGYFKIYSKHTPINLVRDLPQGFSALEPLVDLPIGINITRFQTLLALHRSYLTPGDSSSGWTAGAAAYYVGYLQPRTFLLKYNENGTITDAVDCALDPLSETKCTLKSFTVEKGIYQTSNFRVQPTESIVRFPNITNLCPFGEVFNATRFASVYAWNRKRISNCVADYSVLYNSASFSTFKCYGVSPTKLNDLCFTNVYADSFVIRGDEVRQIAPGQTGKIADYNYKLPDDFTGCVIAWNSNNLDSKVGGNYNYLYRLFRKSNLKPFERDISTEIYQAGSTPCNGVKGFNCYFPLQSYGFQPTNGVGYQPYRVVVLSFELLHAPATVCGPKKSTNLVKNKCVNFNFNGLTGTGVLTESNKKFLPFQQFGRDIADTTDAVRDPQTLEILDITPCSFGGVSVITPGTNTSNQVAVLYQDVNCTEVPVAIHADQLTPTWRVYSTGSNVFQTRAGCLIGAEHVNNSYECDIPIGAGICASYQTQTNSPASVASQSIIAYTMSLGAENSVAYSNNSIAIPTNFTISVTTEILPVSMTKTSVDCTMYICGDSTECSNLLLQYGSFCTQLNRALTGIAVEQDKNTQEVFAQVKQIYKTPPIKDFGGFNFSQILPDPSKPSKRSFIEDLLFNKVTLADAGFIKQYGDCLGDIAARDLICAQKFNGLTVLPPLLTDEMIAQYTSALLAGTITSGWTFGAGAALQIPFAMQMAYRFNGIGVTQNVLYENQKLIANQFNSAIGKIQDSLSSTASALGKLQDVVNQNAQALNTLVKQLSSNFGAISSVLNDILSRLDKVEAEVQIDRLITGRLQSLQTYVTQQLIRAAEIRASANLAATKMSECVLGQSKRVDFCGKGYHLMSFPQSAPHGVVFLHVTYVPAQEKNFTTAPAICHDGKAHFPREGVFVSNGTHWFVTQRNFYEPQIITTDNTFVSGNCDVVIGIVNNTVYDPLQPELDSFKEELDKYFKNHTSPDVDLGDISGINASVVNIQKEIDRLNEVAKNLNESLIDLQELGKYEQYIKWP

SEQ ID NO: 18 - protein, 1196 aa, Unknown
  SARS-CoV-2 Spike protein native ectodomain N487Y mutant
CVNLTTRTQLPPAYTNSFTRGVYYPDKVFRSSVLHSTQDLFLPFFSNVTWFHAIHVSGTNGTKRFDNPVLPFNDGVYFASTEKSNIIRGWIFGTTLDSKTQSLLIVNNATNVVIKVCEFQFCNDPFLGVYYHKNNKSWMESEFRVYSSANNCTFEYVSQPFLMDLEGKQGNFKNLREFVFKNIDGYFKIYSKHTPINLVRDLPQGFSALEPLVDLPIGINITRFQTLLALHRSYLTPGDSSSGWTAGAAAYYVGYLQPRTFLLKYNENGTITDAVDCALDPLSETKCTLKSFTVEKGIYQTSNFRVQPTESIVRFPNITNLCPFGEVFNATRFASVYAWNRKRISNCVADYSVLYNSASFSTFKCYGVSPTKLNDLCFTNVYADSFVIRGDEVRQIAPGQTGKIADYNYKLPDDFTGCVIAWNSNNLDSKVGGNYNYLYRLFRKSNLKPFERDISTEIYQAGSTPCNGVEGFNCYFPLQSYGFQPTYGVGYQPYRVVVLSFELLHAPATVCGPKKSTNLVKNKCVNFNFNGLTGTGVLTESNKKFLPFQQFGRDIADTTDAVRDPQTLEILDITPCSFGGVSVITPGTNTSNQVAVLYQDVNCTEVPVAIHADQLTPTWRVYSTGSNVFQTRAGCLIGAEHVNNSYECDIPIGAGICASYQTQTNSPASVASQSIIAYTMSLGAENSVAYSNNSIAIPTNFTISVTTEILPVSMTKTSVDCTMYICGDSTECSNLLLQYGSFCTQLNRALTGIAVEQDKNTQEVFAQVKQIYKTPPIKDFGGFNFSQILPDPSKPSKRSFIEDLLFNKVTLADAGFIKQYGDCLGDIAARDLICAQKFNGLTVLPPLLTDEMIAQYTSALLAGTITSGWTFGAGAALQIPFAMQMAYRFNGIGVTQNVLYENQKLIANQFNSAIGKIQDSLSSTASALGKLQDVVNQNAQALNTLVKQLSSNFGAISSVLNDILSRLDKVEAEVQIDRLITGRLQSLQTYVTQQLIRAAEIRASANLAATKMSECVLGQSKRVDFCGKGYHLMSFPQSAPHGVVFLHVTYVPAQEKNFTTAPAICHDGKAHFPREGVFVSNGTHWFVTQRNFYEPQIITTDNTFVSGNCDVVIGIVNNTVYDPLQPELDSFKEELDKYFKNHTSPDVDLGDISGINASVVNIQKEIDRLNEVAKNLNESLIDLQELGKYEQYIKWP

SEQ ID NO: 19 - protein, 1196 aa, Unknown
  SARS-CoV-2 Spike protein native ectodomain A556D mutant
CVNLTTRTQLPPAYTNSFTRGVYYPDKVFRSSVLHSTQDLFLPFFSNVTWFHAIHVSGTNGTKRFDNPVLPFNDGVYFASTEKSNIIRGWIFGTTLDSKTQSLLIVNNATNVVIKVCEFQFCNDPFLGVYYHKNNKSWMESEFRVYSSANNCTFEYVSQPFLMDLEGKQGNFKNLREFVFKNIDGYFKIYSKHTPINLVRDLPQGFSALEPLVDLPIGINITRFQTLLALHRSYLTPGDSSSGWTAGAAAYYVGYLQPRTFLLKYNENGTITDAVDCALDPLSETKCTLKSFTVEKGIYQTSNFRVQPTESIVRFPNITNLCPFGEVFNATRFASVYAWNRKRISNCVADYSVLYNSASFSTFKCYGVSPTKLNDLCFTNVYADSFVIRGDEVRQIAPGQTGKIADYNYKLPDDFTGCVIAWNSNNLDSKVGGNYNYLYRLFRKSNLKPFERDISTEIYQAGSTPCNGVEGFNCYFPLQSYGFQPTNGVGYQPYRVVVLSFELLHAPATVCGPKKSTNLVKNKCVNFNFNGLTGTGVLTESNKKFLPFQQFGRDIDDTTDAVRDPQTLEILDITPCSFGGVSVITPGTNTSNQVAVLYQDVNCTEVPVAIHADQLTPTWRVYSTGSNVFQTRAGCLIGAEHVNNSYECDIPIGAGICASYQTQTNSPASVASQSIIAYTMSLGAENSVAYSNNSIAIPTNFTISVTTEILPVSMTKTSVDCTMYICGDSTECSNLLLQYGSFCTQLNRALTGIAVEQDKNTQEVFAQVKQIYKTPPIKDFGGFNFSQILPDPSKPSKRSFIEDLLFNKVTLADAGFIKQYGDCLGDIAARDLICAQKFNGLTVLPPLLTDEMIAQYTSALLAGTITSGWTFGAGAALQIPFAMQMAYRFNGIGVTQNVLYENQKLIANQFNSAIGKIQDSLSSTASALGKLQDVVNQNAQALNTLVKQLSSNFGAISSVLNDILSRLDKVEAEVQIDRLITGRLQSLQTYVTQQLIRAAEIRASANLAATKMSECVLGQSKRVDFCGKGYHLMSFPQSAPHGVVFLHVTYVPAQEKNFTTAPAICHDGKAHFPREGVFVSNGTHWFVTQRNFYEPQIITTDNTFVSGNCDVVIGIVNNTVYDPLQPELDSFKEELDKYFKNHTSPDVDLGDISGINASVVNIQKEIDRLNEVAKNLNESLIDLQELGKYEQYIKWP

SEQ ID NO: 20 - protein, 1196 aa, Unknown
  SARS-CoV-2 Spike protein native ectodomain D600G mutant
CVNLTTRTQLPPAYTNSFTRGVYYPDKVFRSSVLHSTQDLFLPFFSNVTWFHAIHVSGTNGTKRFDNPVLPFNDGVYFASTEKSNIIRGWIFGTTLDSKTQSLLIVNNATNVVIKVCEFQFCNDPFLGVYYHKNNKSWMESEFRVYSSANNCTFEYVSQPFLMDLEGKQGNFKNLREFVFKNIDGYFKIYSKHTPINLVRDLPQGFSALEPLVDLPIGINITRFQTLLALHRSYLTPGDSSSGWTAGAAAYYVGYLQPRTFLLKYNENGTITDAVDCALDPLSETKCTLKSFTVEKGIYQTSNFRVQPTESIVRFPNITNLCPFGEVFNATRFASVYAWNRKRISNCVADYSVLYNSASFSTFKCYGVSPTKLNDLCFTNVYADSFVIRGDEVRQIAPGQTGKIADYNYKLPDDFTGCVIAWNSNNLDSKVGGNYNYLYRLFRKSNLKPFERDISTEIYQAGSTPCNGVEGFNCYFPLQSYGFQPTNGVGYQPYRVVVLSFELLHAPATVCGPKKSTNLVKNKCVNFNFNGLTGTGVLTESNKKFLPFQQFGRDIADTTDAVRDPQTLEILDITPCSFGGVSVITPGTNTSNQVAVLYQGVNCTEVPVAIHADQLTPTWRVYSTGSNVFQTRAGCLIGAEHVNNSYECDIPIGAGICASYQTQTNSPASVASQSIIAYTMSLGAENSVAYSNNSIAIPTNFTISVTTEILPVSMTKTSVDCTMYICGDSTECSNLLLQYGSFCTQLNRALTGIAVEQDKNTQEVFAQVKQIYKTPPIKDFGGFNFSQILPDPSKPSKRSFIEDLLFNKVTLADAGFIKQYGDCLGDIAARDLICAQKFNGLTVLPPLLTDEMIAQYTSALLAGTITSGWTFGAGAALQIPFAMQMAYRFNGIGVTQNVLYENQKLIANQFNSAIGKIQDSLSSTASALGKLQDVVNQNAQALNTLVKQLSSNFGAISSVLNDILSRLDKVEAEVQIDRLITGRLQSLQTYVTQQLIRAAEIRASANLAATKMSECVLGQSKRVDFCGKGYHLMSFPQSAPHGVVFLHVTYVPAQEKNFTTAPAICHDGKAHFPREGVFVSNGTHWFVTQRNFYEPQIITTDNTFVSGNCDVVIGIVNNTVYDPLQPELDSFKEELDKYFKNHTSPDVDLGDISGINASVVNIQKEIDRLNEVAKNLNESLIDLQELGKYEQYIKWP

SEQ ID NO: 21 - protein, 1196 aa, Unknown
  SARS-CoV-2 Spike protein native ectodomain H641Y mutant
CVNLTTRTQLPPAYTNSFTRGVYYPDKVFRSSVLHSTQDLFLPFFSNVTWFHAIHVSGTNGTKRFDNPVLPFNDGVYFASTEKSNIIRGWIFGTTLDSKTQSLLIVNNATNVVIKVCEFQFCNDPFLGVYYHKNNKSWMESEFRVYSSANNCTFEYVSQPFLMDLEGKQGNFKNLREFVFKNIDGYFKIYSKHTPINLVRDLPQGFSALEPLVDLPIGINITRFQTLLALHRSYLTPGDSSSGWTAGAAAYYVGYLQPRTFLLKYNENGTITDAVDCALDPLSETKCTLKSFTVEKGIYQTSNFRVQPTESIVRFPNITNLCPFGEVFNATRFASVYAWNRKRISNCVADYSVLYNSASFSTFKCYGVSPTKLNDLCFTNVYADSFVIRGDEVRQIAPGQTGKIADYNYKLPDDFTGCVIAWNSNNLDSKVGGNYNYLYRLFRKSNLKPFERDISTEIYQAGSTPCNGVEGFNCYFPLQSYGFQPTNGVGYQPYRVVVLSFELLHAPATVCGPKKSTNLVKNKCVNFNFNGLTGTGVLTESNKKFLPFQQFGRDIADTTDAVRDPQTLEILDITPCSFGGVSVITPGTNTSNQVAVLYQDVNCTEVPVAIHADQLTPTWRVYSTGSNVFQTRAGCLIGAEYVNNSYECDIPIGAGICASYQTQTNSPASVASQSIIAYTMSLGAENSVAYSNNSIAIPTNFTISVTTEILPVSMTKTSVDCTMYICGDSTECSNLLLQYGSFCTQLNRALTGIAVEQDKNTQEVFAQVKQIYKTPPIKDFGGFNFSQILPDPSKPSKRSFIEDLLFNKVTLADAGFIKQYGDCLGDIAARDLICAQKFNGLTVLPPLLTDEMIAQYTSALLAGTITSGWTFGAGAALQIPFAMQMAYRFNGIGVTQNVLYENQKLIANQFNSAIGKIQDSLSSTASALGKLQDVVNQNAQALNTLVKQLSSNFGAISSVLNDILSRLDKVEAEVQIDRLITGRLQSLQTYVTQQLIRAAEIRASANLAATKMSECVLGQSKRVDFCGKGYHLMSFPQSAPHGVVFLHVTYVPAQEKNFTTAPAICHDGKAHFPREGVFVSNGTHWFVTQRNFYEPQIITTDNTFVSGNCDVVIGIVNNTVYDPLQPELDSFKEELDKYFKNHTSPDVDLGDISGINASVVNIQKEIDRLNEVAKNLNESLIDLQELGKYEQYIKWP

SEQ ID NO: 22 - protein, 1196 aa, Unknown
  SARS-CoV-2 Spike protein native ectodomain Q663H mutant
CVNLTTRTQLPPAYTNSFTRGVYYPDKVFRSSVLHSTQDLFLPFFSNVTWFHAIHVSGTNGTKRFDNPVLPFNDGVYFASTEKSNIIRGWIFGTTLDSKTQSLLIVNNATNVVIKVCEFQFCNDPFLGVYYHKNNKSWMESEFRVYSSANNCTFEYVSQPFLMDLEGKQGNFKNLREFVFKNIDGYFKIYSKHTPINLVRDLPQGFSALEPLVDLPIGINITRFQTLLALHRSYLTPGDSSSGWTAGAAAYYVGYLQPRTFLLKYNENGTITDAVDCALDPLSETKCTLKSFTVEKGIYQTSNFRVQPTESIVRFPNITNLCPFGEVFNATRFASVYAWNRKRISNCVADYSVLYNSASFSTFKCYGVSPTKLNDLCFTNVYADSFVIRGDEVRQIAPGQTGKIADYNYKLPDDFTGCVIAWNSNNLDSKVGGNYNYLYRLFRKSNLKPFERDISTEIYQAGSTPCNGVEGFNCYFPLQSYGFQPTNGVGYQPYRVVVLSFELLHAPATVCGPKKSTNLVKNKCVNFNFNGLTGTGVLTESNKKFLPFQQFGRDIADTTDAVRDPQTLEILDITPCSFGGVSVITPGTNTSNQVAVLYQDVNCTEVPVAIHADQLTPTWRVYSTGSNVFQTRAGCLIGAEHVNNSYECDIPIGAGICASYQTHTNSPASVASQSIIAYTMSLGAENSVAYSNNSIAIPTNFTISVTTEILPVSMTKTSVDCTMYICGDSTECSNLLLQYGSFCTQLNRALTGIAVEQDKNTQEVFAQVKQIYKTPPIKDFGGFNFSQILPDPSKPSKRSFIEDLLFNKVTLADAGFIKQYGDCLGDIAARDLICAQKFNGLTVLPPLLTDEMIAQYTSALLAGTITSGWTFGAGAALQIPFAMQMAYRFNGIGVTQNVLYENQKLIANQFNSAIGKIQDSLSSTASALGKLQDVVNQNAQALNTLVKQLSSNFGAISSVLNDILSRLDKVEAEVQIDRLITGRLQSLQTYVTQQLIRAAEIRASANLAATKMSECVLGQSKRVDFCGKGYHLMSFPQSAPHGVVFLHVTYVPAQEKNFTTAPAICHDGKAHFPREGVFVSNGTHWFVTQRNFYEPQIITTDNTFVSGNCDVVIGIVNNTVYDPLQPELDSFKEELDKYFKNHTSPDVDLGDISGINASVVNIQKEIDRLNEVAKNLNESLIDLQELGKYEQYIKWP

SEQ ID NO: 23 - protein, 1196 aa, Unknown
  SARS-CoV-2 Spike protein native ectodomain Q663P mutant
CVNLTTRTQLPPAYTNSFTRGVYYPDKVFRSSVLHSTQDLFLPFFSNVTWFHAIHVSGTNGTKRFDNPVLPFNDGVYFASTEKSNIIRGWIFGTTLDSKTQSLLIVNNATNVVIKVCEFQFCNDPFLGVYYHKNNKSWMESEFRVYSSANNCTFEYVSQPFLMDLEGKQGNFKNLREFVFKNIDGYFKIYSKHTPINLVRDLPQGFSALEPLVDLPIGINITRFQTLLALHRSYLTPGDSSSGWTAGAAAYYVGYLQPRTFLLKYNENGTITDAVDCALDPLSETKCTLKSFTVEKGIYQTSNFRVQPTESIVRFPNITNLCPFGEVFNATRFASVYAWNRKRISNCVADYSVLYNSASFSTFKCYGVSPTKLNDLCFTNVYADSFVIRGDEVRQIAPGQTGKIADYNYKLPDDFTGCVIAWNSNNLDSKVGGNYNYLYRLFRKSNLKPFERDISTEIYQAGSTPCNGVEGFNCYFPLQSYGFQPTNGVGYQPYRVVVLSFELLHAPATVCGPKKSTNLVKNKCVNFNFNGLTGTGVLTESNKKFLPFQQFGRDIADTTDAVRDPQTLEILDITPCSFGGVSVITPGTNTSNQVAVLYQDVNCTEVPVAIHADQLTPTWRVYSTGSNVFQTRAGCLIGAEHVNNSYECDIPIGAGICASYQTPTNSPASVASQSIIAYTMSLGAENSVAYSNNSIAIPTNFTISVTTEILPVSMTKTSVDCTMYICGDSTECSNLLLQYGSFCTQLNRALTGIAVEQDKNTQEVFAQVKQIYKTPPIKDFGGFNFSQILPDPSKPSKRSFIEDLLFNKVTLADAGFIKQYGDCLGDIAARDLICAQKFNGLTVLPPLLTDEMIAQYTSALLAGTITSGWTFGAGAALQIPFAMQMAYRFNGIGVTQNVLYENQKLIANQFNSAIGKIQDSLSSTASALGKLQDVVNQNAQALNTLVKQLSSNFGAISSVLNDILSRLDKVEAEVQIDRLITGRLQSLQTYVTQQLIRAAEIRASANLAATKMSECVLGQSKRVDFCGKGYHLMSFPQSAPHGVVFLHVTYVPAQEKNFTTAPAICHDGKAHFPREGVFVSNGTHWFVTQRNFYEPQIITTDNTFVSGNCDVVIGIVNNTVYDPLQPELDSFKEELDKYFKNHTSPDVDLGDISGINASVVNIQKEIDRLNEVAKNLNESLIDLQELGKYEQYIKWP

SEQ ID NO: 24 - protein, 1196 aa, Unknown
  SARS-CoV-2 Spike protein native ectodomain P667H mutant
CVNLTTRTQLPPAYTNSFTRGVYYPDKVFRSSVLHSTQDLFLPFFSNVTWFHAIHVSGTNGTKRFDNPVLPFNDGVYFASTEKSNIIRGWIFGTTLDSKTQSLLIVNNATNVVIKVCEFQFCNDPFLGVYYHKNNKSWMESEFRVYSSANNCTFEYVSQPFLMDLEGKQGNFKNLREFVFKNIDGYFKIYSKHTPINLVRDLPQGFSALEPLVDLPIGINITRFQTLLALHRSYLTPGDSSSGWTAGAAAYYVGYLQPRTFLLKYNENGTITDAVDCALDPLSETKCTLKSFTVEKGIYQTSNFRVQPTESIVRFPNITNLCPFGEVFNATRFASVYAWNRKRISNCVADYSVLYNSASFSTFKCYGVSPTKLNDLCFTNVYADSFVIRGDEVRQIAPGQTGKIADYNYKLPDDFTGCVIAWNSNNLDSKVGGNYNYLYRLFRKSNLKPFERDISTEIYQAGSTPCNGVEGFNCYFPLQSYGFQPTNGVGYQPYRVVVLSFELLHAPATVCGPKKSTNLVKNKCVNFNFNGLTGTGVLTESNKKFLPFQQFGRDIADTTDAVRDPQTLEILDITPCSFGGVSVITPGTNTSNQVAVLYQDVNCTEVPVAIHADQLTPTWRVYSTGSNVFQTRAGCLIGAEHVNNSYECDIPIGAGICASYQTQTNSHASVASQSIIAYTMSLGAENSVAYSNNSIAIPTNFTISVTTEILPVSMTKTSVDCTMYICGDSTECSNLLLQYGSFCTQLNRALTGIAVEQDKNTQEVFAQVKQIYKTPPIKDFGGFNFSQILPDPSKPSKRSFIEDLLFNKVTLADAGFIKQYGDCLGDIAARDLICAQKFNGLTVLPPLLTDEMIAQYTSALLAGTITSGWTFGAGAALQIPFAMQMAYRFNGIGVTQNVLYENQKLIANQFNSAIGKIQDSLSSTASALGKLQDVVNQNAQALNTLVKQLSSNFGAISSVLNDILSRLDKVEAEVQIDRLITGRLQSLQTYVTQQLIRAAEIRASANLAATKMSECVLGQSKRVDFCGKGYHLMSFPQSAPHGVVFLHVTYVPAQEKNFTTAPAICHDGKAHFPREGVFVSNGTHWFVTQRNFYEPQIITTDNTFVSGNCDVVIGIVNNTVYDPLQPELDSFKEELDKYFKNHTSPDVDLGDISGINASVVNIQKEIDRLNEVAKNLNESLIDLQELGKYEQYIKWP

SEQ ID NO: 25 - protein, 1196 aa, Unknown
  SARS-CoV-2 Spike protein native ectodomain A684V mutant
CVNLTTRTQLPPAYTNSFTRGVYYPDKVFRSSVLHSTQDLFLPFFSNVTWFHAIHVSGTNGTKRFDNPVLPFNDGVYFASTEKSNIIRGWIFGTTLDSKTQSLLIVNNATNVVIKVCEFQFCNDPFLGVYYHKNNKSWMESEFRVYSSANNCTFEYVSQPFLMDLEGKQGNFKNLREFVFKNIDGYFKIYSKHTPINLVRDLPQGFSALEPLVDLPIGINITRFQTLLALHRSYLTPGDSSSGWTAGAAAYYVGYLQPRTFLLKYNENGTITDAVDCALDPLSETKCTLKSFTVEKGIYQTSNFRVQPTESIVRFPNITNLCPFGEVFNATRFASVYAWNRKRISNCVADYSVLYNSASFSTFKCYGVSPTKLNDLCFTNVYADSFVIRGDEVRQIAPGQTGKIADYNYKLPDDFTGCVIAWNSNNLDSKVGGNYNYLYRLFRKSNLKPFERDISTEIYQAGSTPCNGVEGFNCYFPLQSYGFQPTNGVGYQPYRVVVLSFELLHAPATVCGPKKSTNLVKNKCVNFNFNGLTGTGVLTESNKKFLPFQQFGRDIADTTDAVRDPQTLEILDITPCSFGGVSVITPGTNTSNQVAVLYQDVNCTEVPVAIHADQLTPTWRVYSTGSNVFQTRAGCLIGAEHVNNSYECDIPIGAGICASYQTQTNSPASVASQSIIAYTMSLGVENSVAYSNNSIAIPTNFTISVTTEILPVSMTKTSVDCTMYICGDSTECSNLLLQYGSFCTQLNRALTGIAVEQDKNTQEVFAQVKQIYKTPPIKDFGGFNFSQILPDPSKPSKRSFIEDLLFNKVTLADAGFIKQYGDCLGDIAARDLICAQKFNGLTVLPPLLTDEMIAQYTSALLAGTITSGWTFGAGAALQIPFAMQMAYRFNGIGVTQNVLYENQKLIANQFNSAIGKIQDSLSSTASALGKLQDVVNQNAQALNTLVKQLSSNFGAISSVLNDILSRLDKVEAEVQIDRLITGRLQSLQTYVTQQLIRAAEIRASANLAATKMSECVLGQSKRVDFCGKGYHLMSFPQSAPHGVVFLHVTYVPAQEKNFTTAPAICHDGKAHFPREGVFVSNGTHWFVTQRNFYEPQIITTDNTFVSGNCDVVIGIVNNTVYDPLQPELDSFKEELDKYFKNHTSPDVDLGDISGINASVVNIQKEIDRLNEVAKNLNESLIDLQELGKYEQYIKWP

SEQ ID NO: 26 - protein, 1196 aa, Unknown
  SARS-CoV-2 Spike protein native ectodomain T699I mutant
CVNLTTRTQLPPAYTNSFTRGVYYPDKVFRSSVLHSTQDLFLPFFSNVTWFHAIHVSGTNGTKRFDNPVLPFNDGVYFASTEKSNIIRGWIFGTTLDSKTQSLLIVNNATNVVIKVCEFQFCNDPFLGVYYHKNNKSWMESEFRVYSSANNCTFEYVSQPFLMDLEGKQGNFKNLREFVFKNIDGYFKIYSKHTPINLVRDLPQGFSALEPLVDLPIGINITRFQTLLALHRSYLTPGDSSSGWTAGAAAYYVGYLQPRTFLLKYNENGTITDAVDCALDPLSETKCTLKSFTVEKGIYQTSNFRVQPTESIVRFPNITNLCPFGEVFNATRFASVYAWNRKRISNCVADYSVLYNSASFSTFKCYGVSPTKLNDLCFTNVYADSFVIRGDEVRQIAPGQTGKIADYNYKLPDDFTGCVIAWNSNNLDSKVGGNYNYLYRLFRKSNLKPFERDISTEIYQAGSTPCNGVEGFNCYFPLQSYGFQPTNGVGYQPYRVVVLSFELLHAPATVCGPKKSTNLVKNKCVNFNFNGLTGTGVLTESNKKFLPFQQFGRDIADTTDAVRDPQTLEILDITPCSFGGVSVITPGTNTSNQVAVLYQDVNCTEVPVAIHADQLTPTWRVYSTGSNVFQTRAGCLIGAEHVNNSYECDIPIGAGICASYQTQTNSPASVASQSIIAYTMSLGAENSVAYSNNSIAIPINFTISVTTEILPVSMTKTSVDCTMYICGDSTECSNLLLQYGSFCTQLNRALTGIAVEQDKNTQEVFAQVKQIYKTPPIKDFGGFNFSQILPDPSKPSKRSFIEDLLFNKVTLADAGFIKQYGDCLGDIAARDLICAQKFNGLTVLPPLLTDEMIAQYTSALLAGTITSGWTFGAGAALQIPFAMQMAYRFNGIGVTQNVLYENQKLIANQFNSAIGKIQDSLSSTASALGKLQDVVNQNAQALNTLVKQLSSNFGAISSVLNDILSRLDKVEAEVQIDRLITGRLQSLQTYVTQQLIRAAEIRASANLAATKMSECVLGQSKRVDFCGKGYHLMSFPQSAPHGVVFLHVTYVPAQEKNFTTAPAICHDGKAHFPREGVFVSNGTHWFVTQRNFYEPQIITTDNTFVSGNCDVVIGIVNNTVYDPLQPELDSFKEELDKYFKNHTSPDVDLGDISGINASVVNIQKEIDRLNEVAKNLNESLIDLQELGKYEQYIKWP

SEQ ID NO: 27 - protein, 1196 aa, Unknown
  SARS-CoV-2 Spike protein native ectodomain S965A mutant
CVNLTTRTQLPPAYTNSFTRGVYYPDKVFRSSVLHSTQDLFLPFFSNVTWFHAIHVSGTNGTKRFDNPVLPFNDGVYFASTEKSNIIRGWIFGTTLDSKTQSLLIVNNATNVVIKVCEFQFCNDPFLGVYYHKNNKSWMESEFRVYSSANNCTFEYVSQPFLMDLEGKQGNFKNLREFVFKNIDGYFKIYSKHTPINLVRDLPQGFSALEPLVDLPIGINITRFQTLLALHRSYLTPGDSSSGWTAGAAAYYVGYLQPRTFLLKYNENGTITDAVDCALDPLSETKCTLKSFTVEKGIYQTSNFRVQPTESIVRFPNITNLCPFGEVFNATRFASVYAWNRKRISNCVADYSVLYNSASFSTFKCYGVSPTKLNDLCFTNVYADSFVIRGDEVRQIAPGQTGKIADYNYKLPDDFTGCVIAWNSNNLDSKVGGNYNYLYRLFRKSNLKPFERDISTEIYQAGSTPCNGVEGFNCYFPLQSYGFQPTNGVGYQPYRVVVLSFELLHAPATVCGPKKSTNLVKNKCVNFNFNGLTGTGVLTESNKKFLPFQQFGRDIADTTDAVRDPQTLEILDITPCSFGGVSVITPGTNTSNQVAVLYQDVNCTEVPVAIHADQLTPTWRVYSTGSNVFQTRAGCLIGAEHVNNSYECDIPIGAGICASYQTQTNSPASVASQSIIAYTMSLGAENSVAYSNNSIAIPTNFTISVTTEILPVSMTKTSVDCTMYICGDSTECSNLLLQYGSFCTQLNRALTGIAVEQDKNTQEVFAQVKQIYKTPPIKDFGGFNFSQILPDPSKPSKRSFIEDLLFNKVTLADAGFIKQYGDCLGDIAARDLICAQKFNGLTVLPPLLTDEMIAQYTSALLAGTITSGWTFGAGAALQIPFAMQMAYRFNGIGVTQNVLYENQKLIANQFNSAIGKIQDSLSSTASALGKLQDVVNQNAQALNTLVKQLSSNFGAISSVLNDILARLDKVEAEVQIDRLITGRLQSLQTYVTQQLIRAAEIRASANLAATKMSECVLGQSKRVDFCGKGYHLMSFPQSAPHGVVFLHVTYVPAQEKNFTTAPAICHDGKAHFPREGVFVSNGTHWFVTQRNFYEPQIITTDNTFVSGNCDVVIGIVNNTVYDPLQPELDSFKEELDKYFKNHTSPDVDLGDISGINASVVNIQKEIDRLNEVAKNLNESLIDLQELGKYEQYIKWP

SEQ ID NO: 28 - protein, 1196 aa, Unknown
  SARS-CoV-2 Spike protein native ectodomain T1010I mutant
CVNLTTRTQLPPAYTNSFTRGVYYPDKVFRSSVLHSTQDLFLPFFSNVTWFHAIHVSGTNGTKRFDNPVLPFNDGVYFASTEKSNIIRGWIFGTTLDSKTQSLLIVNNATNVVIKVCEFQFCNDPFLGVYYHKNNKSWMESEFRVYSSANNCTFEYVSQPFLMDLEGKQGNFKNLREFVFKNIDGYFKIYSKHTPINLVRDLPQGFSALEPLVDLPIGINITRFQTLLALHRSYLTPGDSSSGWTAGAAAYYVGYLQPRTFLLKYNENGTITDAVDCALDPLSETKCTLKSFTVEKGIYQTSNFRVQPTESIVRFPNITNLCPFGEVFNATRFASVYAWNRKRISNCVADYSVLYNSASFSTFKCYGVSPTKLNDLCFTNVYADSFVIRGDEVRQIAPGQTGKIADYNYKLPDDFTGCVIAWNSNNLDSKVGGNYNYLYRLFRKSNLKPFERDISTEIYQAGSTPCNGVEGFNCYFPLQSYGFQPTNGVGYQPYRVVVLSFELLHAPATVCGPKKSTNLVKNKCVNFNFNGLTGTGVLTESNKKFLPFQQFGRDIADTTDAVRDPQTLEILDITPCSFGGVSVITPGTNTSNQVAVLYQDVNCTEVPVAIHADQLTPTWRVYSTGSNVFQTRAGCLIGAEHVNNSYECDIPIGAGICASYQTQTNSPASVASQSIIAYTMSLGAENSVAYSNNSIAIPTNFTISVTTEILPVSMTKTSVDCTMYICGDSTECSNLLLQYGSFCTQLNRALTGIAVEQDKNTQEVFAQVKQIYKTPPIKDFGGFNFSQILPDPSKPSKRSFIEDLLFNKVTLADAGFIKQYGDCLGDIAARDLICAQKFNGLTVLPPLLTDEMIAQYTSALLAGTITSGWTFGAGAALQIPFAMQMAYRFNGIGVTQNVLYENQKLIANQFNSAIGKIQDSLSSTASALGKLQDVVNQNAQALNTLVKQLSSNFGAISSVLNDILSRLDKVEAEVQIDRLITGRLQSLQTYVTQQLIRAAEIRASANLAAIKMSECVLGQSKRVDFCGKGYHLMSFPQSAPHGVVFLHVTYVPAQEKNFTTAPAICHDGKAHFPREGVFVSNGTHWFVTQRNFYEPQIITTDNTFVSGNCDVVIGIVNNTVYDPLQPELDSFKEELDKYFKNHTSPDVDLGDISGINASVVNIQKEIDRLNEVAKNLNESLIDLQELGKYEQYIKWP

SEQ ID NO: 29 - protein, 1196 aa, Unknown
  SARS-CoV-2 Spike protein native ectodomain D1101H mutant
CVNLTTRTQLPPAYTNSFTRGVYYPDKVFRSSVLHSTQDLFLPFFSNVTWFHAIHVSGTNGTKRFDNPVLPFNDGVYFASTEKSNIIRGWIFGTTLDSKTQSLLIVNNATNVVIKVCEFQFCNDPFLGVYYHKNNKSWMESEFRVYSSANNCTFEYVSQPFLMDLEGKQGNFKNLREFVFKNIDGYFKIYSKHTPINLVRDLPQGFSALEPLVDLPIGINITRFQTLLALHRSYLTPGDSSSGWTAGAAAYYVGYLQPRTFLLKYNENGTITDAVDCALDPLSETKCTLKSFTVEKGIYQTSNFRVQPTESIVRFPNITNLCPFGEVFNATRFASVYAWNRKRISNCVADYSVLYNSASFSTFKCYGVSPTKLNDLCFTNVYADSFVIRGDEVRQIAPGQTGKIADYNYKLPDDFTGCVIAWNSNNLDSKVGGNYNYLYRLFRKSNLKPFERDISTEIYQAGSTPCNGVEGFNCYFPLQSYGFQPTNGVGYQPYRVVVLSFELLHAPATVCGPKKSTNLVKNKCVNFNFNGLTGTGVLTESNKKFLPFQQFGRDIADTTDAVRDPQTLEILDITPCSFGGVSVITPGTNTSNQVAVLYQDVNCTEVPVAIHADQLTPTWRVYSTGSNVFQTRAGCLIGAEHVNNSYECDIPIGAGICASYQTQTNSPASVASQSIIAYTMSLGAENSVAYSNNSIAIPTNFTISVTTEILPVSMTKTSVDCTMYICGDSTECSNLLLQYGSFCTQLNRALTGIAVEQDKNTQEVFAQVKQIYKTPPIKDFGGFNFSQILPDPSKPSKRSFIEDLLFNKVTLADAGFIKQYGDCLGDIAARDLICAQKFNGLTVLPPLLTDEMIAQYTSALLAGTITSGWTFGAGAALQIPFAMQMAYRFNGIGVTQNVLYENQKLIANQFNSAIGKIQDSLSSTASALGKLQDVVNQNAQALNTLVKQLSSNFGAISSVLNDILSRLDKVEAEVQIDRLITGRLQSLQTYVTQQLIRAAEIRASANLAATKMSECVLGQSKRVDFCGKGYHLMSFPQSAPHGVVFLHVTYVPAQEKNFTTAPAICHDGKAHFPREGVFVSNGTHWFVTQRNFYEPQIITTHNTFVSGNCDVVIGIVNNTVYDPLQPELDSFKEELDKYFKNHTSPDVDLGDISGINASVVNIQKEIDRLNEVAKNLNESLIDLQELGKYEQYIKWP

SEQ ID NO: 30 - protein, 401 aa, Artificial Sequence
  Recombinant Dengue virus 2 E-glycoprotein (His tag)
MTMRCIGMSNRDFVEGVSGGSWVDIVLEHGSCVTTMAKNKPTLDFELIKTEAKQPATLRKYCIEAKLTNTTTESRCPTQGEPSLNEEQDKRFVCKHSMVDRGWGNGCGLFGKGGIVTCAMFRCKKNMEGKVVQPENLEYTIVITPHSGEEHAVGNDTGKHGKEIKITPQSSTTEAELTGYGTVTMECSPRTGLDFNEMVLLQMENKAWLVHRQWFLDLPLPWLPGADTQGSNWIQKETLVTFKNPHAKKQDVVVLGSQEGAMHTALTGATEIQMSSGNLLFTGHLKCRLRMDKLQLKGMSYSMCTGKFKVVKEIAETQHGTIVIRVQYEGDGSPCKIPFEIMDLEKRHVLGRLITVNPIVTEKDSPVNIEAEPPFGDSYIIIGVEPGQLKLNWFKKGSSIG

SEQ ID NO: 31 - DNA, 19 bp, Artificial Sequence
  GAPDH-For 5' primer
gaaggtgaaggtcggagtc

SEQ ID NO: 32 - DNA, 20 bp, Artificial Sequence
  GAPDH-Rev 5' primer
gaagatggtgatgggatttc

SEQ ID NO: 33 - DNA, 24 bp, Artificial Sequence
  CoV-2 Leader_For 5' primer
tcccaggtaacaaaccaaccaact

SEQ ID NO: 34 - DNA, 20 bp, Artificial Sequence
  CoV-2 Orf7a_Rev 5'  primer
aaatggtgaattgccctcgt

SEQ ID NO: 35 - protein, 20 aa, Artificial Sequence
  GP64 secretion signal sequence
MVSAIVLYVLLAAAAHSAFA